European Patent Application EP 4 782 003 A1, published July 29, 2026. Title: 신규한 파킨슨 병 치료제. Applicant: 주식회사 스탠드업테라퓨틱스. Application WO. The sequence listing filed with the application follows.

SEQUENCE LISTING (15 sequences)

SEQ ID NO: 1 - protein, 873 aa, Homo sapiens
  source 1..873: note = Human wild type NDST3 protein
MSFIMKLHRHFQRTVILLATFCMVSIIISAYYLYSGYKQENELSETASEVDCGDLQHLPYQLMEVKAMKLFDASRTDPTVLVFVESQYSSLGQDIIMILESSRFQYHIEIAPGKGDLPVLIDKMKGKYILIIYENILKYINMDSWNRSLLDKYCVEYGVGVIGFHKTSEKSVQSFQLKGFPFSIYGNLAVKDCCINPHSPLIRVTKSSKLEKGSLPGTDWTVFQINHSAYQPVIFAKVKTPENLSPSISKGAFYATIIHDLGLHDGIQRVLFGNNLNFWLHKLIFIDAISFLSGKRLTLSLDRYILVDIDDIFVGKEGTRMNTNDVKALLDTQNLLRAQITNFTFNLGFSGKFYHTGTEEEDEGDDCLLGSVDEFWWFPHMWSHMQPHLFHNESSLVEQMILNKKFALEHGIPTDMGYAVAPHHSGVYPVHVQLYEAWKKVWNIKITSTEEYPHLKPARYRRGFIHKNIMVLPRQTCGLFTHTIFYKEYPGGPKELDKSIQGGELFFTVVLNPISIFMTHLSNYGNDRLGLYTFVNLANFVKSWTNLRLQTLPPVQLAHKYFELFPDQKDPLWQNPCDDKRHRDIWSKEKTCDRLPKFLVIGPQKTGTTALYLFLVMHPSILSNSPSPKTFEEVQFFNRNNYHRGIDWYMDFFPVPSNVTTDFLFEKSANYFHSEEAPKRAASLVPKAKIITILIDPSDRAYSWYQHQRSHEDPAALKFSFYEVISAGPRAPSELRALQKRCLVPGWYASHIERWLVYFPPFQLLIIDGQQLRTDPATVMDEVQKFLGVLPHYNYSEALTFDSHKGFWCQLLEEGKTKCLGKSKGRKYPPMDSDSRTFLSSYYRDHNVELSKLLHKLGQPLPSWLRQELQKVR

SEQ ID NO: 2 - protein, 899 aa, Homo sapiens
  source 1..899: note = Human NDST3 protein isoform X1
MSFIMKLHRHFQRTVILLATFCMVSIIISAYYLYSGYKQENELSETASEVDCGDLQHLPYQLMEVKAMKLFDASRTDPTVLVFVESQYSSLGQDIIMILESSRFQYHIEIAPGKGDLPVLIDKMKGKYILIIYENILKYINMDSWNRSLLDKYCVEYGVGVIGFHKTSEKSVQSFQLKGFPFSIYGNLAVKDCCINPHSPLIRVTKSSKLEKGSLPGTDWTVFQINHSAYQPVIFAKVKTPENLSPSISKGAFYATIIHDLGLHDGIQRVLFGNNLNFWLHKLIFIDAISFLSGKRLTLSLDRYILVDIDDIFVGKEGTRMNTNDVKALLDTQNLLRAQITNFTFNLGFSGKFYHTGTEEEDEGDDCLLGSVDEFWWFPHMWSHMQPHLFHNESSLVEQMILNKKFALEHGIPTDMGYAVAPHHSGVYPVHVQLYEAWKKVWNIKITSTEEYPHLKPARYRRGFIHKNIMVLPRQTCGLFTHTIFYKEYPGGPKELDKSIQGGELFFTVVLNPISIFMTHLSNYGNDRLGLYTFVNLANFVKSWTNLRLQTLPPVQLAHKYFELFPDQKDPLWQNPCDDKRHRDIWSKEKTCDRLPKFLVIGPQKTGTTALYLFLVMHPSILSNSPSPKTFEEVQFFNRNNYHRGIDWYMDFFPVPSNVTTDFLFEKSANYFHSEEAPKRAASLVPKAKIITILIDPSDRAYSWYQHQRSHEDPAALKFSFYEVISAGPRAPSELRALQKRCLVPGWYASHIERWLVYFPPFQLLIIDGQQLRTDPATVMDEVQKFLGVLPHYNYSEALTFDSHKGFWCQLLEEGKTKCLGKSKGRKYPPMDSDDISVKLLSRSQRGTLKAAAQTGSASAILAETGAAESKIALRENLRLHRPCRTHLFQSFQKLPKGS

SEQ ID NO: 3 - protein, 524 aa, Homo sapiens
  source 1..524: note = Human NDST3 protein isoform X3
MSFIMKLHRHFQRTVILLATFCMVSIIISAYYLYSGYKQENELSETASEVDCGDLQHLPYQLMEVKAMKLFDASRTDPTVLVFVESQYSSLGQDIIMILESSRFQYHIEIAPGKGDLPVLIDKMKGKYILIIYENILKYINMDSWNRSLLDKYCVEYGVGVIGFHKTSEKSVQSFQLKGFPFSIYGNLAVKDCCINPHSPLIRVTKSSKLEKGSLPGTDWTVFQINHSAYQPVIFAKVKTPENLSPSISKGAFYATIIHDLGLHDGIQRVLFGNNLNFWLHKLIFIDAISFLSGKRLTLSLDRYILVDIDDIFVGKEGTRMNTNDVKALLDTQNLLRAQITNFTFNLGFSGKFYHTGTEEEDEGDDCLLGSVDEFWWFPHMWSHMQPHLFHNESSLVEQMILNKKFALEHGIPTDMGYAVAPHHSGVYPVHVQLYEAWKKVWNIKITSTEEYPHLKPARYRRGFIHKNIMVLPRQTCGLFTHTIFYKEYPGGPKELDKSIQGGELFFTVVLNPFIIDCKLNRQS

SEQ ID NO: 4 - protein, 519 aa, Homo sapiens
  source 1..519: note = Human NDST3 protein isoform X4
MWSHMQPHLFHNESSLVEQMILNKKFALEHGIPTDMGYAVAPHHSGVYPVHVQLYEAWKKVWNIKITSTEEYPHLKPARYRRGFIHKNIMVLPRQTCGLFTHTIFYKEYPGGPKELDKSIQGGELFFTVVLNPISIFMTHLSNYGNDRLGLYTFVNLANFVKSWTNLRLQTLPPVQLAHKYFELFPDQKDPLWQNPCDDKRHRDIWSKEKTCDRLPKFLVIGPQKTGTTALYLFLVMHPSILSNSPSPKTFEEVQFFNRNNYHRGIDWYMDFFPVPSNVTTDFLFEKSANYFHSEEAPKRAASLVPKAKIITILIDPSDRAYSWYQHQRSHEDPAALKFSFYEVISAGPRAPSELRALQKRCLVPGWYASHIERWLVYFPPFQLLIIDGQQLRTDPATVMDEVQKFLGVLPHYNYSEALTFDSHKGFWCQLLEEGKTKCLGKSKGRKYPPMDSDDISVKLLSRSQRGTLKAAAQTGSASAILAETGAAESKIALRENLRLHRPCRTHLFQSFQKLPKGS

SEQ ID NO: 5 - protein, 516 aa, Homo sapiens
  source 1..516: note = Human NDST3 protein isoform X5
MSFIMKLHRHFQRTVILLATFCMVSIIISAYYLYSGYKQENELSETASEVDCGDLQHLPYQLMEVKAMKLFDASRTDPTVLVFVESQYSSLGQDIIMILESSRFQYHIEIAPGKGDLPVLIDKMKGKYILIIYENILKYINMDSWNRSLLDKYCVEYGVGVIGFHKTSEKSVQSFQLKGFPFSIYGNLAVKDCCINPHSPLIRVTKSSKLEKGSLPGTDWTVFQINHSAYQPVIFAKVKTPENLSPSISKGAFYATIIHDLGLHDGIQRVLFGNNLNFWLHKLIFIDAISFLSGKRLTLSLDRYILVDIDDIFVGKEGTRMNTNDVKALLDTQNLLRAQITNFTFNLGFSGKFYHTGTEEEDEGDDCLLGSVDEFWWFPHMWSHMQPHLFHNESSLVEQMILNKKFALEHGIPTDMGYAVAPHHSGVYPVHVQLYEAWKKVWNIKITSTEEYPHLKPARYRRGFIHKNIMVLPRQTCGLFTHTIFYKEYPGGPKELDKSIQGGELFFTVVLNPKMR

SEQ ID NO: 6 - protein, 484 aa, Homo sapiens
  source 1..484: note = Human NDST3 protein isoform X6
MGYAVAPHHSGVYPVHVQLYEAWKKVWNIKITSTEEYPHLKPARYRRGFIHKNIMVLPRQTCGLFTHTIFYKEYPGGPKELDKSIQGGELFFTVVLNPISIFMTHLSNYGNDRLGLYTFVNLANFVKSWTNLRLQTLPPVQLAHKYFELFPDQKDPLWQNPCDDKRHRDIWSKEKTCDRLPKFLVIGPQKTGTTALYLFLVMHPSILSNSPSPKTFEEVQFFNRNNYHRGIDWYMDFFPVPSNVTTDFLFEKSANYFHSEEAPKRAASLVPKAKIITILIDPSDRAYSWYQHQRSHEDPAALKFSFYEVISAGPRAPSELRALQKRCLVPGWYASHIERWLVYFPPFQLLIIDGQQLRTDPATVMDEVQKFLGVLPHYNYSEALTFDSHKGFWCQLLEEGKTKCLGKSKGRKYPPMDSDDISVKLLSRSQRGTLKAAAQTGSASAILAETGAAESKIALRENLRLHRPCRTHLFQSFQKLPKGS

SEQ ID NO: 7 - DNA, 2622 bp, synthetic construct
  source 1..2622: mol_type = other DNA; note = CDS encoding human wild type NDST3 protein
atgagttttatcatgaagcttcacagacactttcaaagaacagtcattctgcttgccactttttgtatggtgagcattattatttctgcttactacctgtacagtggctacaaacaggaaaatgaactctctgagacggcttcagaagttgactgtggcgacctccaacacctaccatatcaactaatggaagtgaaagcaatgaagctttttgatgcctcaaggacagaccccacagtcctagtatttgtagagagccagtactcatctcttggtcaagacatcattatgattctagaatcaagtagattccagtatcacattgaaattgcccctggaaagggagatctcccagtgcttatagacaaaatgaaaggcaaatacattctcattatttatgagaatattttaaagtatataaatatggattcctggaatcgaagccttctagataaatactgtgtagaatatggtgtgggtgtcattggattccacaaaactagtgagaagagtgtacagagctttcagttaaaaggtttccctttttccatatatggaaatcttgcagtaaaagattgttgtattaatcctcattctccattgattcgtgtgaccaaatcttccaagcttgaaaaaggttctttacctggaactgactggacagtttttcagattaatcattcagcctatcaaccagtaatatttgccaaagtaaagaccccagaaaacctttctccttccatctctaaaggtgctttttatgccactattatacatgacctggggcttcatgatggaattcaaagggttctttttggcaacaacttgaacttttggctgcacaagctcatcttcatagatgccatctccttcttatcagggaagaggctgacattgtccttggacaggtacattcttgtggatattgatgatatatttgtgggaaaagagggaacaagaatgaacaccaatgatgtaaaggccctgcttgatactcagaatcttttgcgtgcacaaatcacaaattttacattcaacctgggattttcagggaaattttaccatacaggaactgaagaggaagatgaaggagatgactgtctgttggggtctgtggatgagttctggtggtttcctcacatgtggagccatatgcagccccacctcttccacaatgagtcatctttggtggagcagatgattctcaacaaaaaatttgccttagagcacggcattccaacggacatgggctacgctgtggcccctcaccattcgggcgtctaccctgtacatgttcagctttatgaggcctggaagaaggtctggaatattaaaatcaccagcactgaagaatatccacatctgaagccagctagataccggaggggttttatccacaaaaacatcatggttctcccaagacaaacctgtgggcttttcactcacaccattttctacaaagaatatccagggggtcctaaagagctggataagagtatccaaggaggagaacttttcttcactgtcgtcctcaaccctatcagcattttcatgacccatttgtccaactatgggaatgaccgactgggattatatacatttgttaatctggccaactttgtgaagagctggaccaacctgcgacttcagactctgcctccagtacaactggcccacaagtattttgagctgtttcctgatcagaaagaccctctctggcagaatccttgcgatgacaaacgccacagagacatttggtctaaagaaaaaacttgtgatcgcttaccaaaattcttggtaataggaccccagaaaactggtaccactgctttgtatttgttcctggttatgcatccttccatccttagtaactcccccagcccaaaaacctttgaggaggtacagttctttaatagaaataactaccacagggggattgattggtatatggatttcttcccagtcccatctaatgtcactaccgactttttgtttgagaagagtgccaattacttccactcagaggaagcccctaaaagagctgcttctctggttcccaaagccaagattatcaccattctcattgacccttcagaccgagcatactcctggtaccagcatcagcgatcacatgaagaccctgcagctctgaagtttagcttctacgaagtgatctcagcagggccccgtgcaccctcggagctcagagccttgcagaagagatgtttggtcccggggtggtatgccagccacatcgagagatggcttgtttatttccccccatttcagttgctaattattgatgggcaacaactaagaactgatcctgctacagtgatggatgaagtacagaagtttctaggagtcttgcctcattataattactcagaagctttaacgtttgattctcataaaggtttctggtgtcagttactggaagaaggtaaaacaaaatgccttggaaagagcaaaggaagaaaataccctccaatggattctgatagcaggacatttctgtcaagctactatcgagatcacaacgtggaactctcaaagctgctgcacaaactgggtcagcctctgccatcctggctgagacaggagctgcagaaagtaagatag

SEQ ID NO: 8 - DNA, 204 bp, synthetic construct
  source 1..204: mol_type = other DNA; note = CMV promoter
gtgatgcggttttggcagtacatcaatgggcgtggatagcggtttgactcacggggatttccaagtctccaccccattgacgtcaatgggagtttgttttggcaccaaaatcaacgggactttccaaaatgtcgtaacaactccgccccattgacgcaaatgggcggtaggcgtgtacggtgggaggtctatataagcagagct

SEQ ID NO: 9 - DNA, 514 bp, synthetic construct
  source 1..514: mol_type = other DNA; note = M13 ori
acgcgccctgtagcggcgcattaagcgcggcgggtgtggtggttacgcgcagcgtgaccgctacacttgccagcgccctagcgcccgctcctttcgctttcttcccttcctttctcgccacgttcgccggctttccccgtcaagctctaaatcgggggctccctttagggttccgatttagtgctttacggcacctcgaccccaaaaaacttgattagggtgatggttcacgtagtgggccatcgccctgatagacggtttttcgccctttgacgttggagtccacgttctttaatagtggactcttgttccaaactggaacaacactcaaccctatctcggtctattcttttgatttataagggattttgccgatttcggcctattggttaaaaaatgagctgatttaacaaaaatttaacgcgaattttaacaaaatattaacgcttacaatttaaatatttgcttatacaatcttcctgtttttggggcttttctgattatcaaccggggt

SEQ ID NO: 10 - DNA, 795 bp, synthetic construct
  source 1..795: mol_type = other DNA; note = NeoR/KanR
atgattgaacaagatggattgcacgcaggttctccggccgcttgggtggagaggctattcggctatgactgggcacaacagacaatcggctgctctgatgccgccgtgttccggctgtcagcgcaggggcgcccggttctttttgtcaagaccgacctgtccggtgccctgaatgaactgcaagacgaggcagcgcggctatcgtggctggccacgacgggcgttccttgcgcagctgtgctcgacgttgtcactgaagcgggaagggactggctgctattgggcgaagtgccggggcaggatctcctgtcatctcaccttgctcctgccgagaaagtatccatcatggctgatgcaatgcggcggctgcatacgcttgatccggctacctgcccattcgaccaccaagcgaaacatcgcatcgagcgagcacgtactcggatggaagccggtcttgtcgatcaggatgatctggacgaagagcatcaggggctcgcgccagccgaactgttcgccaggctcaaggcgagcatgcccgacggcgaggatctcgtcgtgacccatggcgatgcctgcttgccgaatatcatggtggaaaatggccgcttttctggattcatcgactgtggccggctgggtgtggcggaccgctatcaggacatagcgttggctacccgtgatattgctgaagagcttggcggcgaatgggctgaccgcttcctcgtgctttacggtatcgccgctcccgattcgcagcgcatcgccttctatcgccttcttgacgagttcttctga

SEQ ID NO: 11 - DNA, 762 bp, synthetic construct
  source 1..762: mol_type = other DNA; note = NG2 promoter
ttgagctgcactttcgtcctccatgaaatgggggaggggatgctcctcacccaccttgcaaggttattttgaggcaaatgtcatggcgggactgagaattcttctgccctgcgaggaaatccagacatctctcccttacagacagggagactgaggtgaggcccttccaggcagagaaggtcactgttgcagccatgggcagtgccccacaggacctcgggtggtgcctctggagtctggagaagttcctaggggacctccgaggcaaagcagcccaaaagccgcctgtgagggtggctggtgtctgtccttcctcctaaggctggagtgtgcctgtggaggggtctcctgaactcccgcaaaggcagaaaggagggaagtaggggctgggacagttcatgcctcctccctgagggggtctcccgggctcggctcttggggccagagttcagggtgtctgggcctctctatgactttgttctaagtctttagggtggggctggggtctggcccagctgcaagggccccctcacccctgccccagagaggaacagccccgcacgggccctttaagaaggttgagggtgggggcaggtgggggagtccaagcctgaaacccgagcgggcgcgcgggtctgcgcctgccccgcccccggagttaagtgcgcggacacccggagccggcccgcgcccaggagcagagccgcgctcgctccactcagctcccagctcccaggactccgctggctcctcgcaagtcct

SEQ ID NO: 12 - DNA, 20 bp, synthetic construct
  source 1..20: mol_type = other DNA; note = mGAPDH-F primer
tgatgggtgtgaaccacgag

SEQ ID NO: 13 - DNA, 20 bp, synthetic construct
  source 1..20: mol_type = other DNA; note = mGAPDH-R primer
ggtcatgagcccttccacaa

SEQ ID NO: 14 - DNA, 20 bp, synthetic construct
  source 1..20: mol_type = other DNA; note = mNdst3-F primer
ggaaacgaccgactgggatt

SEQ ID NO: 15 - DNA, 20 bp, synthetic construct
  source 1..20: mol_type = other DNA; note = mNdst3-R primer
tacttgtgagccagctgagc